European Patent Specification EP 3 578 194 B1, published July 26, 2023. Title: Injectable composition for prevention of depilation or improvement of hair growth. Applicant: Keramedix inc. The sequence listing filed with the application follows.

SEQUENCE LISTING (16 sequences)

SEQ ID NO: 1 - DNA, 20 bp, Artificial Sequence
  beta-catenin primerF
tgcagttcgccttcactatg

SEQ ID NO: 2 - DNA, 20 bp, Artificial Sequence
  beta-catenin primerR
ctgcacaaacaatggaatgg

SEQ ID NO: 3 - DNA, 19 bp, Artificial Sequence
  KRT5 primerF
accagtacccgcatctgca

SEQ ID NO: 4 - DNA, 18 bp, Artificial Sequence
  KRT5 primerR
tgttccgtggcctcttcg

SEQ ID NO: 5 - DNA, 20 bp, Artificial Sequence
  MSX2 primerF
ccgccaagacatatgagccc

SEQ ID NO: 6 - DNA, 20 bp, Artificial Sequence
  MSX2 primerR
acctgggtctctgtgaggtt

SEQ ID NO: 7 - DNA, 20 bp, Artificial Sequence
  ITGA6 primerF
agctgtgcttgctctacctg

SEQ ID NO: 8 - DNA, 20 bp, Artificial Sequence
  ITGA6 primerR
ccggggtctccatatttccg

SEQ ID NO: 9 - DNA, 20 bp, Artificial Sequence
  FOXN1 primerF
agtggtgctgggatgttctg

SEQ ID NO: 10 - DNA, 20 bp, Artificial Sequence
  FOXN1 primerR
atagtgtgaggagcccaggt

SEQ ID NO: 11 - DNA, 20 bp, Artificial Sequence
  CD10 primerF
ctttagtgcccagcagtcca

SEQ ID NO: 12 - DNA, 20 bp, Artificial Sequence
  CD10 primerR
gagtccaccagtcaacgagg

SEQ ID NO: 13 - DNA, 20 bp, Artificial Sequence
  beta-actin primerF
gtcaggcagctcgtagctct

SEQ ID NO: 14 - DNA, 20 bp, Artificial Sequence
  beta-actin primerR
tcgtgcgtgacattaaggag

SEQ ID NO: 15 - DNA, 19 bp, Artificial Sequence
  Sox-9 primerF
accagtacccgcatctgca

SEQ ID NO: 16 - DNA, 18 bp, Artificial Sequence
  Sox-9 primerR
tgttccgtggcctcttcg